European Patent Application EP 4 299 582 A1, published January 3, 2024. Title: VSV vector-encoded HCV envelope proteins E1/E2 as vaccines against Hepatitis C virus. Applicant: TWINCORE, Zentrum für Experimentelle und Klinische Infektionsforschung GmbH. Application EP. The sequence listing filed with the application follows.

SEQUENCE LISTING (16 sequences)

SEQ ID NO: 1 - protein, 192 aa, Hepatitis C virus
AEVKNISTGYMVTNDCTNDSITWQLQAAVLHVPGCVPCEKVGNASQCWIPVSPNVAVQRPGALTQGLRTHIDMVVMSATLCSALYVGDLCGGVMLAAQMFIVSPQHHWFVQDCNCSIYPGTITGHRMAWDMMMNWSPTATMILAYAMRVPEVIIDIISGAHWGVMFGLAYFSMQGAWAKVVVILLLAAGVDA

SEQ ID NO: 2 - protein, 367 aa, Hepatitis C virus
  VARIANT 1..27: note = HVR1
RTHTVGGSAAQTTGRLTSLFDMGPRQKIQLVNTNGSWHINRTALNCNDSLHTGFIASLFYTHSFNSSGCPERMSACRSIEAFRVGWGALQYEDNVTNPEDMRPYCWHYPPRQCGVVSAKTVCGPVYCFTPSPVVVGTTDRLGAPTYTWGENETDVFLLNSTRPPLGSWFGCTWMNSSGYTKTCGAPPCRTRADFNASTDLLCPTDCFRKHPDTTYLKCGSGPWLTPRCLIDYPYRLWHYPCTVNYTIFKIRMYVGGVEHRLTAACNFTRGDRCNLEDRDRSQLSPLLHSTTEWAILPCSYSDLPALSTGLLHLHQNIVDVQFMYGLSPALTKYIVRWEWVILLFLLLADARVCACLWMLILLGQAEA

SEQ ID NO: 3 - protein, 60 aa, Hepatitis C virus
DLMGYIPVVGAPLGGVARALAHGVRVLEDGVNFATGNLPGCSFSIFLLALLSCITTPVSA

SEQ ID NO: 4 - protein, 192 aa, Hepatitis C virus
VQVKNTSTMYQVTNDCPNSSIVWQLKDAVLHVPGCVPCEQVNNMSRCWLPVTPNVAISQPGALTRGLRTHIDIIVMSATLCSALYVGDVCGGVMIASQAFVVSPQMHHFVQDCNCSIYPGHVTGHRMAWDMMMNWSPTATMIMAYAVRIPELALEIIAGGHWGVLFGLAYFSLQGAWAKVVVILLLFAGVEA

SEQ ID NO: 5 - protein, 367 aa, Hepatitis C virus
  VARIANT 1..27: note = HVR1
HTHVVGGSVAQGARGFTGLFSPGSQQNIQLINTNGSWHINRTALNCNDSLNTGFLASLFYTHKFNSSGCPERMSACKGIEAFRIGWGVLEHEENVTNDEDMRPYCWHYPPKPCGIVPARTVCGPVYCFTPSPVVVGTTDRRGVPTYTWGENETDVFLLNSTRPPGGSWFGCTWMNSTGYTKTCGAPPCRIRADFNASTDLLCPTDCFRKHPDATYGKCGAGPWLTPKCLVDYPYRLWHYPCTVNFTIFKIRMYVGGVEHRLQAACNFSRGDRCNLEDRDRSQLSPLLHSTTEWAILPCTFSDMPALSTGLLHLHQNIVDVQYLYGLSPALTKYMVKWEWVVLLFLLLADARICACLWMLILMGQAEA

SEQ ID NO: 6 - protein, 60 aa, Hepatitis C virus; identical to SEQ ID NO: 3

SEQ ID NO: 7 - protein, 192 aa, Hepatitis C virus
VPYRNASGVYHVTNDCPNSSIVYEAEDLILHAPGCVPCVRQGNVSRCWVQITPTLSAPSLGAVTAPLRRAVDYLAGGAALCSALYVGDACGAVFLVGQMFTYSPRRHNVVQDCNCSIYSGHITGHRMAWDMMMNWSPTTALVMAQLLRIPQVVIDIIAGAHWGVLFAAAYYASAANWAKVVLVLFLFAGVDA

SEQ ID NO: 8 - protein, 364 aa, Hepatitis C virus
  VARIANT 1..27: note = 1..27
STRTVGGSAAQGARGLASLFTPGPQQNLQLINTNGSWHINRTALNCNDSLQTGFVAGLLYYHKFNSTGCPQRMASCRPLAAFDQGWGTISYAAVSGPSDDKPYCWHYPPRPCGIVPARGVCGPVYCFTPSPVVVGTTDRKGNPTYSWGENETDIFLLNNTRPPTGNWFGCTWMNSTGFVKTCGAPPCNLGPTGNNSLKCPTDCFRKHPDATYTKCGSGPWLTPRCLVHYPYRLWHYPCTLNYTIFKVRMYIGGLEHRLEVACNWTRGERCDLEDRDRAELSPLLHTTTQWAILPCSFTPTPALSTGLIHLHQNIVDTQYLYGLSSSIVSWAVKWEYIVLAFLLLADARICTCLWIMLLVCQAEA

SEQ ID NO: 9 - protein, 60 aa, Hepatitis C virus
DLMGYIPLVGGPVGGVARALAHGVRVLEDGVNYATGNLPGCSFSIFILALLSCLTVPTSA

SEQ ID NO: 10 - RNA, 1857 nt, synthetic construct
  source 1..1857: mol_type = other RNA
gacctcatggggtacatccctgtcgtgggcgccccgctcggcggcgtcgccagagctctcgcgcatggcgtgagagtcctggaggacggggttaattttgcaacagggaacttacccggttgctccttttctatcttcttgctggccctgctgtcctgcatcaccaccccggtctccgctgccgaagtgaagaacatcagtaccggctacatggtgactaacgactgcaccaatgacagcattacctggcagctccaggctgctgtcctccacgtccccgggtgcgtcccgtgcgagaaagtggggaatgcatctcagtgctggataccggtctcaccgaatgtggccgtgcagcggcccggcgccctcacgcagggcttgcggacgcacatcgacatggttgtgatgtccgccacgctctgctctgccctctacgtgggggacctctgcggtggggtgatgctcgcagcccaaatgttcattgtctcgccgcagcaccactggtttgtccaagactgcaattgctccatctaccctggtaccatcactggacaccgcatggcatgggacatgatgatgaactggtcgcccacggctaccatgatcttggcgtacgcgatgcgtgtccccgaggtcattatagacatcattagcggggctcattggggcgtcatgttcggcttggcctacttctctatgcagggagcgtgggcgaaagtcgttgtcatccttctgttggccgccggggtggacgcgcgcacccatactgttgggggttctgccgcgcagaccaccgggcgcctcaccagcttatttgacatgggccccaggcagaaaatccagctcgttaacaccaatggcagctggcacatcaaccgcaccgccctgaactgcaatgactccttgcacaccggctttatcgcgtctctgttctacacccacagcttcaactcgtcaggatgtcccgaacgcatgtccgcctgccgcagtatcgaggccttccgggtgggatggggcgccttgcaatatgaggataatgtcaccaatccagaggatatgagaccctattgctggcactacccaccaaggcagtgtggcgtggtctccgcgaagactgtgtgtggcccagtgtactgtttcacccccagcccagtggtagtgggcacgaccgacaggcttggagcgcccacttacacgtggggggagaatgagacagatgtcttcctattgaacagcactcgaccaccgctggggtcatggttcggctgcacgtggatgaactcttctggctacaccaagacttgcggcgcaccaccctgccgtactagagctgacttcaacgccagcacggacctgttgtgccccacggactgttttaggaagcatcctgataccacttacctcaaatgcggctctgggccctggctcacgccaaggtgcctgatcgactacccctacaggctctggcattacccctgcacagttaactataccatcttcaaaataaggatgtatgtgggaggggttgagcacaggctcacggctgcatgcaatttcactcgtggggatcgttgcaacttggaggacagagacagaagtcaactgtctcctttgttgcactccaccacggaatgggccattttaccttgctcttactcggacctgcccgccttgtcgactggtcttctccacctccaccaaaacatcgtggacgtacaattcatgtatggcctatcacctgccctcacaaaatacatcgtccgatgggagtgggtaatactcttattcctgctcttagcggacgccagggtttgcgcctgcttatggatgctcatcttgttgggccaggccgaagca

SEQ ID NO: 11 - RNA, 1857 nt, synthetic construct
  source 1..1857: mol_type = other RNA
gacctcatggggtacatccctgtcgtgggcgccccgctcggcggcgtcgccagagctctcgcgcatggcgtgagagtcctggaggacggggttaattttgcaacagggaacttacccggttgctccttttctatcttcttgctggccctgctgtcctgcatcaccaccccggtctccgctgtgcaagtcaagaacaccagcacaatgtaccaggtgactaatgactgtcctaactccagtatagtctggcagcttaaggatgccgtccttcacgtccctgggtgtgtcccctgtgagcaagtgaacaacatgtcccggtgttggttaccggtcactcccaatgtggccatcagccaacctggggccctcactaggggcttgcggacgcacattgacattattgtgatgtccgccactctgtgctcagccctctatgtgggggatgtgtgtggcggggtgatgatagcctctcaggctttcgttgtctcgccgcaaatgcaccacttcgtccaggactgcaactgttccatctatccgggccatgtcacgggacatcgtatggcatgggatatgatgatgaattggtcgccgactgccaccatgatcatggcatatgcggtgcgtatccccgagcttgccttggagatcatcgctggcggccattggggtgtgctgtttggcctagcttacttctccttgcaaggagcgtgggcgaaggtcgtcgtcatcctcctgctgtttgcaggagtggaggcgcatacccacgtagttgggggcagcgtagcccagggcgcccggggctttactggcctgttctccccggggtcccagcagaacattcagcttattaacaccaatggtagttggcacattaaccgcacggccctcaattgcaatgatagccttaacaccggcttccttgcttctctgttctacacccataagttcaactcctcaggctgtccggagcgcatgtctgcctgtaagggcattgaggcgttccggatagggtggggtgtcttggaacatgaggagaacgtgaccaacgatgaggacatgaggccctactgctggcactacccgcctaaaccttgtggtatcgttccagctcgaacggtatgtggcccagtctactgcttcacccccagtccagtagtagtgggcactaccgacaggcgcggtgtgcccacttacacctggggggaaaatgagacagatgtctttctgctcaacagcacccgcccccctgggggcagttggtttgggtgcacgtggatgaactccactggctacaccaagacctgcggcgcaccaccttgccgcatcagagcagatttcaatgccagcacagacctactatgccccacagactgctttaggaagcatcccgatgcgacctatggcaagtgtggggctggaccctggttaactccaaaatgtctggttgactacccctacaggctgtggcactacccgtgcacagtcaatttcaccatctttaagatcaggatgtacgtggggggagtcgaacacaggctacaagcagcgtgtaacttcagtcgtggagaccgctgtaatctggaggacagggataggagccaattaagcccacttctgcattccaccactgagtgggccatcctaccctgcactttttcagatatgccggctttgtcaacagggttgctgcatcttcaccagaatatcgtggacgtgcagtacttgtatggtctgtcaccggccctcacaaaatacatggtcaaatgggaatgggtggtcctgctcttcctgctcttagcagatgctaggatctgcgcatgtctttggatgctcatcctgatgggccaggctgaggca

SEQ ID NO: 12 - RNA, 1848 nt, synthetic construct
  source 1..1848: mol_type = other RNA
gacctcatggggtacatcccgctcgtaggcggccccgttgggggcgtcgcaagggctctcgcacacggtgtgagggtccttgaggacggggtaaactatgcaacagggaatttacccggttgctctttctctatctttatccttgcacttctttcatgcctgactgtcccgacctctgccgttccctaccgaaatgcctctggggtttatcatgtcaccaatgattgcccaaactcttctatcgtctatgaggctgaagacctgatcttacacgcacctggttgcgtgccctgtgttaggcagggtaatgtcagtaggtgctgggtccagatcacccccacactgtcagccccgagcctcggagcggtcacggctcctcttcggagggccgttgactacttagcggggggggctgccctttgctccgcgttatacgtcggagacgcgtgcggggcagtgtttttggtaggtcaaatgttcacctatagccctcgccggcataatgttgtgcaggactgcaactgttccatttacagtggccacatcaccggccaccggatggcatgggacatgatgatgaattggtcacctacaacagctttggtgatggcccagttgttacggattccccaggtggtcattgacatcattgccggggcccactggggggtcttgttcgccgccgcatactacgcgtcggcggctaactgggccaaggttgtgctggtcctgtttctgtttgcgggggtcgatgccagcacccgcactgtgggtggtagtgcggcccaaggcgcgcgcgggctcgcttcacttttcacccctgggccgcagcagaacttgcagctcataaataccaacgggagctggcacatcaacagaactgcccttaactgtaatgacagcctccagactgggtttgtagccggcctcctgtattatcacaagttcaactccactgggtgtccgcagcggatggctagctgtaggcccctcgccgcattcgaccagggctggggaactatcagctatgccgccgtgtcgggccccagtgatgacaagccctattgctggcactaccccccacgcccgtgcggaatagtgccagcgcgaggtgtctgcggtccggtctattgttttacacctagcccggtggtcgtcggcaccacagaccgcaaggggaatcccacttacagttggggcgaaaatgagactgacatctttctcttgaacaacacgaggccccctactggcaactggtttggctgcacctggatgaattccacagggtttgtcaagacttgcggggctccaccctgcaacttagggcctacaggcaacaatagccttaagtgtcctactgattgcttccgcaagcacccagacgccacctacaccaagtgtgggtcaggaccctggctcactccccggtgtctggtgcattacccttaccggttgtggcattacccgtgcaccctaaattacaccatcttcaaggtgcgcatgtacattgggggcctcgagcacaggctcgaggtggcatgcaactggacccgtggtgagcggtgtgatcttgaagacagggatagggccgagctgagcccgctcctacataccaccacgcagtgggccatattgccgtgctctttcacacccacacccgctcttagcactggtctcatacacttacatcaaaatatagtagacacccagtatctttacggtctgagctccagcatcgtctcgtgggccgttaagtgggagtacatagtgctggccttcttattacttgctgatgcccgtatttgtacttgcctatggatcatgctcctggtttgtcaggccgaagcg

SEQ ID NO: 13 - RNA, 14579 nt, synthetic construct
  source 1..14579: mol_type = other RNA
ctaaattgtaagcgttaatattttgttaaaattcgcgttaaatttttgttaaatcagctcattttttaaccaataggccgaaatcggcaaaatcccttataaatcaaaagaatagaccgagatagggttgagtgttgttccagtttggaacaagagtccactattaaagaacgtggactccaacgtcaaagggcgaaaaaccgtctatcagggcgatggcccactacgtgaaccatcaccctaatcaagttttttggggtcgaggtgccgtaaagcactaaatcggaaccctaaagggagcccccgatttagagcttgacggggaaagccggcgaacgtggcgagaaaggaagggaagaaagcgaaaggagcgggcgctagggcgctggcaagtgtagcggtcacgctgcgcgtaaccaccacacccgccgcgcttaatgcgccgctacagggcgcgtcccattcgccattcaggctgcgcaactgttgggaagggcgatcggtgcgggcctcttcgctattacgccagctggcgaaagggggatgtgctgcaaggcgattaagttgggtaacgccagggttttcccagtcacgacgttgtaaaacgacggccagtgagcgcgcgtaatacgactcactatagggacgaagacaaacaaaccattattatcattaaaaggctcaggagaaactttaacagtaatcaaaatgtctgttacagtcaagagaatcattgacaacacagtcgtagttccaaaacttcctgcaaatgaggatccagtggaatacccggcagattacttcagaaaatcaaaggagattcctctttacatcaatactacaaaaagtttgtcagatctaagaggatatgtctaccaaggcctcaaatccggaaatgtatcaatcatacatgtcaacagctacttgtatggagcattaaaggacatccggggtaagttggataaagattggtcaagtttcggaataaacatcgggaaagcaggggatacaatcggaatatttgaccttgtatccttgaaagccctggacggcgtacttccagatggagtatcggatgcttccagaaccagcgcagatgacaaatggttgcctttgtatctacttggcttatacagagtgggcagaacacaaatgcctgaatacagaaaaaagctcatggatgggctgacaaatcaatgcaaaatgatcaatgaacagtttgaacctcttgtgccagaaggtcgtgacatttttgatgtgtggggaaatgacagtaattacacaaaaattgtcgctgcagtggacatgttcttccacatgttcaaaaaacatgaatgtgcctcgttcagatacggaactattgtttccagattcaaagattgtgctgcattggcaacatttggacacctctgcaaaataaccggaatgtctacagaagatgtaacgacctggatcttgaaccgagaagttgcagatgaaatggtccaaatgatgcttccaggccaagaaattgacaaggccgattcatacatgccttatttgatcgactttggattgtcttctaagtctccatattcttccgtcaaaaaccctgccttccacttctgggggcaattgacagctcttctgctcagatccaccagagcaaggaatgcccgacagcctgatgacattgagtatacatctcttactacagcaggtttgttgtacgcttatgcagtaggatcctctgccgacttggcacaacagttttgtgttggagataacaaatacactccagatgatagtaccggaggattgacgactaatgcaccgccacaaggcagagatgtggtcgaatggctcggatggtttgaagatcaaaacagaaaaccgactcctgatatgatgcagtatgcgaaaagagcagtcatgtcactgcaaggcctaagagagaagacaattggcaagtatgctaagtcagaatttgacaaatgaccctataattctcagatcacctattatatattatgctacatatgaaaaaaactaacagatatcatggataatctcacaaaagttcgtgagtatctcaagtcctattctcgtctggatcaggcggtaggagagatagatgagatcgaagcacaacgagctgaaaagtccaattatgagttgttccaagaggatggagtggaagagcatactaagccctcttattttcaggcagcagatgattctgacacagaatctgaaccagaaattgaagacaatcaaggcttgtatgcaccagatccagaagctgagcaagttgaaggctttatacaggggcctttagatgactatgcagatgaggaagtggatgttgtatttacttcggactggaaacagcctgagcttgaatctgacgagcatggaaagaccttacggttgacatcgccagagggtttaagtggagagcagaaatcccagtggctttcgacgattaaagcagtcgtgcaaagtgccaaatactggaatctggcagagtgcacatttgaagcatcgggagaaggggtcattatgaaggagcgccagataactccggatgtatataaggtcactccagtgatgaacacacatccgtcccaatcagaagcagtatcagatgtttggtctctctcaaagacatccatgactttccaacccaagaaagcaagtcttcagcctctcaccatatccttggatgaattgttctcatctagaggagagttcatctctgtcggaggtgacggacgaatgtctcataaagaggccatcctgctcggcctgagatacaaaaagttgtacaatcaggcgagagtcaaatattctctgtagactatgaaaaaaagtaacagatatcacgatctaagtgttatcccaatccattcatcatgagttccttaaagaagattctcggtctgaaggggaaaggtaagaaatctaagaaattagggatcgcaccacccccttatgaagaggacactagcatggagtatgctccgagcgctccaattgacaaatcctattttggagttgacgagatggacacctatgatccgaatcaattaagatatgagaaattcttctttacagtgaaaatgacggttagatctaatcgtccgttcagaacatactcagatgtggcagccgctgtatcccattgggatcacatgtacatcggaatggcagggaaacgtcccttctacaaaatcttggcttttttgggttcttctaatctaaaggccactccagcggtattggcagatcaaggtcaaccagagtatcacgctcactgcgaaggcagggcttatttgccacataggatggggaagacccctcccatgctcaatgtaccagagcacttcagaagaccattcaatataggtctttacaagggaacgattgagctcacaatgaccatctacgatgatgagtcactggaagcagctcctatgatctgggatcatttcaattcttccaaattttctgatttcagagagaaggccttaatgtttggcctgattgtcgagaaaaaggcatctggagcgtgggtcctggactctatcggccacttcaaatgagctagtctaacttctagcttctgaacaatccccggtttactcagtctcccctaattccagcctctcgaacaactaatatcctgtcttttctatccctatgaaaaaaactaacagagatcgatctgtttacgcgtaaaatggacctcatggggtacatccctgtcgtgggcgccccgctcggcggcgtcgccagagctctcgcgcatggcgtgagagtcctggaggacggggttaattttgcaacagggaacttacccggttgctccttttctatcttcttgctggccctgctgtcctgcatcaccaccccggtctccgctgccgaagtgaagaacatcagtaccggctacatggtgactaacgactgcaccaatgacagcattacctggcagctccaggctgctgtcctccacgtccccgggtgcgtcccgtgcgagaaagtggggaatgcatctcagtgctggataccggtctcaccgaatgtggccgtgcagcggcccggcgccctcacgcagggcttgcggacgcacatcgacatggttgtgatgtccgccacgctctgctctgccctctacgtgggggacctctgcggtggggtgatgctcgcagcccaaatgttcattgtctcgccgcagcaccactggtttgtccaagactgcaattgctccatctaccctggtaccatcactggacaccgcatggcatgggacatgatgatgaactggtcgcccacggctaccatgatcttggcgtacgcgatgcgtgtccccgaggtcattatagacatcattagcggggctcattggggcgtcatgttcggcttggcctacttctctatgcagggagcgtgggcgaaagtcgttgtcatccttctgttggccgccggggtggacgcgcgcacccatactgttgggggttctgccgcgcagaccaccgggcgcctcaccagcttatttgacatgggccccaggcagaaaatccagctcgttaacaccaatggcagctggcacatcaaccgcaccgccctgaactgcaatgactccttgcacaccggctttatcgcgtctctgttctacacccacagcttcaactcgtcaggatgtcccgaacgcatgtccgcctgccgcagtatcgaggccttccgggtgggatggggcgccttgcaatatgaggataatgtcaccaatccagaggatatgagaccctattgctggcactacccaccaaggcagtgtggcgtggtctccgcgaagactgtgtgtggcccagtgtactgtttcacccccagcccagtggtagtgggcacgaccgacaggcttggagcgcccacttacacgtggggggagaatgagacagatgtcttcctattgaacagcactcgaccaccgctggggtcatggttcggctgcacgtggatgaactcttctggctacaccaagacttgcggcgcaccaccctgccgtactagagctgacttcaacgccagcacggacctgttgtgccccacggactgttttaggaagcatcctgataccacttacctcaaatgcggctctgggccctggctcacgccaaggtgcctgatcgactacccctacaggctctggcattacccctgcacagttaactataccatcttcaaaataaggatgtatgtgggaggggttgagcacaggctcacggctgcatgcaatttcactcgtggggatcgttgcaacttggaggacagagacagaagtcaactgtctcctttgttgcactccaccacggaatgggccattttaccttgctcttactcggacctgcccgccttgtcgactggtcttctccacctccaccaaaacatcgtggacgtacaattcatgtatggcctatcacctgccctcacaaaatacatcgtccgatgggagtgggtaatactcttattcctgctcttagcggacgccagggtttgcgcctgcttatggatgctcatcttgttgggccaggccgaagcataagctagccagattcttcatgtttggaccaaatcaacttgtgataccatgctcaaagaggcctcaattatatttgagtttttaatttttatgaaaaaaactaacagcaatcatggaagtccacgattttgagaccgacgagttcaatgatttcaatgaagatgactatgccacaagagaattcctgaatcccgatgagcgcatgacgtacttgaatcatgctgattacaacctgaattctcctctaattagtgatgatattgacaatttaatcaggaaattcaattctcttccaattccctcgatgtgggatagtaagaactgggatggagttcttgagatgttaacgtcatgtcaagccaatcccatcccaacatctcagatgcataaatggatgggaagttggttaatgtctgataatcatgatgccagtcaagggtatagttttttacatgaagtggacaaagaggcagaaataacatttgacgtggtggagaccttcatccgcggctggggcaacaaaccaattgaatacatcaaaaaggaaagatggactgactcattcaaaattctcgcttatttgtgtcaaaagtttttggacttacacaagttgacattaatcttaaatgctgtctctgaggtggaattgctcaacttggcgaggactttcaaaggcaaagtcagaagaagttctcatggaacgaacatatgcaggattagggttcccagcttgggtcctacttttatttcagaaggatgggcttacttcaagaaacttgatattctaatggaccgaaactttctgttaatggtcaaagatgtgattatagggaggatgcaaacggtgctatccatggtatgtagaatagacaacctgttctcagagcaagacatcttctcccttctaaatatctacagaattggagataaaattgtggagaggcagggaaatttttcttatgacttgattaaaatggtggaaccgatatgcaacttgaagctgatgaaattagcaagagaatcaaggcctttagtcccacaattccctcattttgaaaatcatatcaagacttctgttgatgaaggggcaaaaattgaccgaggtataagattcctccatgatcagataatgagtgtgaaaacagtggatctcacactggtgatttatggatcgttcagacattggggtcatccttttatagattattacactggactagaaaaattacattcccaagtaaccatgaagaaagatattgatgtgtcatatgcaaaagcacttgcaagtgatttagctcggattgttctatttcaacagttcaatgatcataaaaagtggttcgtgaatggagacttgctccctcatgatcatccctttaaaagtcatgttaaagaaaatacatggcccacagctgctcaagttcaagattttggagataaatggcatgaacttccgctgattaaatgttttgaaatacccgacttactagacccatcgataatatactctgacaaaagtcattcaatgaataggtcagaggtgttgaaacatgtccgaatgaatccgaacactcctatccctagtaaaaaggtgttgcagactatgttggacacaaaggctaccaattggaaagaatttcttaaagagattgatgagaagggcttagatgatgatgatctaattattggtcttaaaggaaaggagagggaactgaagttggcaggtagatttttctccctaatgtcttggaaattgcgagaatactttgtaattaccgaatatttgataaagactcatttcgtccctatgtttaaaggcctgacaatggcggacgatctaactgcagtcattaaaaagatgttagattcctcatccggccaaggattgaagtcatatgaggcaatttgcatagccaatcacattgattacgaaaaatggaataaccaccaaaggaagttatcaaacggcccagtgttccgagttatgggccagttcttaggttatccatccttaatcgagagaactcatgaattttttgagaaaagtcttatatactacaatggaagaccagacttgatgcgtgttcacaacaacacactgatcaattcaacctcccaacgagtttgttggcaaggacaagagggtggactggaaggtctacggcaaaaaggatggagtatcctcaatctactggttattcaaagagaggctaaaatcagaaacactgctgtcaaagtcttggcacaaggtgataatcaagttatttgcacacagtataaaacgaagaaatcgagaaacgttgtagaattacagggtgctctcaatcaaatggtttctaataatgagaaaattatgactgcaatcaaaatagggacagggaagttaggacttttgataaatgacgatgagactatgcaatctgcagattacttgaattatggaaaaataccgattttccgtggagtgattagagggttagagaccaagagatggtcacgagtgacttgtgtcaccaatgaccaaatacccacttgtgctaatataatgagctcagtttccacaaatgctctcaccgtagctcattttgctgagaacccaatcaatgccatgatacagtacaattattttgggacatttgctagactcttgttgatgatgcatgatcctgctcttcgtcaatcattgtatgaagttcaagataagataccgggcttgcacagttctactttcaaatacgccatgttgtatttggacccttccattggaggagtgtcgggcatgtctttgtccaggtttttgattagagccttcccagatcccgtaacagaaagtctctcattctggagattcatccatgtacatgctcgaagtgagcatctgaaggagatgagtgcagtatttggaaaccccgagatagccaagtttcgaataactcacatagacaagctagtagaagatccaacctctctgaacatcgctatgggaatgagtccagcgaacttgttaaagactgaggttaaaaaatgcttaatcgaatcaagacaaaccatcaggaaccaggtgattaaggatgcaaccatatatttgtatcatgaagaggatcggctcagaagtttcttatggtcaataaatcctctgttccctagatttttaagtgaattcaaatcaggcacttttttgggagtcgcagacgggctcatcagtctatttcaaaattctcgtactattcggaactcctttaagaaaaagtatcatagggaattggatgatttgattgtgaggagtgaggtatcctctttgacacatttagggaaacttcatttgagaaggggatcatgtaaaatgtggacatgttcagctactcatgctgacacattaagatacaaatcctggggccgtacagttattgggacaactgtaccccatccattagaaatgttgggtccacaacatcgaaaagagactccttgtgcaccatgtaacacatcagggttcaattatgtttctgtgcattgtccagacgggatccatgacgtctttagttcacggggaccattgcctgcttatctagggtctaaaacatctgaatctacatctattttgcagccttgggaaagggaaagcaaagtcccactgattaaaagagctacacgtcttagagatgctatctcttggtttgttgaacccgactctaaactagcaatgactatactttctaacatccactctttaacaggcgaagaatggaccaaaaggcagcatgggttcaaaagaacagggtctgcccttcataggttttcgacatctcggatgagccatggtgggttcgcatctcagagcactgcagcattgaccaggttgatggcaactacagacaccatgagggatctgggagatcagaatttcgactttttattccaagcaacgttgctctatgctcaaattaccaccactgttgcaagagacggatggatcaccagttgtacagatcattatcatattgcctgtaagtcctgtttgagacccatagaagagatcaccctggactcaagtatggactacacgcccccagatgtatcccatgtgctgaagacatggaggaatggggaaggttcgtggggacaagagataaaacagatctatcctttagaagggaattggaagaatttagcacctgctgagcaatcctatcaagtcggcagatgtataggttttctatatggagacttggcgtatagaaaatctactcatgccgaggacagttctctatttcctctatctatacaaggtcgtattagaggtcgaggtttcttaaaagggttgctagacggattaatgagagcaagttgctgccaagtaatacaccggagaagtctggctcatttgaagaggccggccaacgcagtgtacggaggtttgatttacttgattgataaattgagtgtatcacctccattcctttctcttactagatcaggacctattagagacgaattagaaacgattccccacaagatcccaacctcctatccgacaagcaaccgtgatatgggggtgattgtcagaaattacttcaaataccaatgccgtctaattgaaaagggaaaatacagatcacattattcacaattatggttattctcagatgtcttatccatagacttcattggaccattctctatttccaccaccctcttgcaaatcctatacaagccatttttatctgggaaagataagaatgagttgagagagctggcaaatctttcttcattgctaagatcaggagaggggtgggaagacatacatgtgaaattcttcaccaaggacatattattgtgtccagaggaaatcagacatgcttgcaagttcgggattgctaaggataataataaagacatgagctatcccccttggggaagggaatccagagggacaattacaacaatccctgtttattatacgaccaccccttacccaaagatgctagagatgcctccaagaatccaaaatcccctgctgtccggaatcaggttgggccaattaccaactggcgctcattataaaattcggagtatattacatggaatgggaatccattacagggacttcttgagttgtggagacggctccggagggatgactgctgcattactacgagaaaatgtgcatagcagaggaatattcaatagtctgttagaattatcagggtcagtcatgcgaggcgcctctcctgagccccccagtgccctagaaactttaggaggagataaatcgagatgtgtaaatggtgaaacatgttgggaatatccatctgacttatgtgacccaaggacttgggactatttcctccgactcaaagcaggcttggggcttcaaattgatttaattgtaatggatatggaagttcgggattcttctactagcctgaaaattgagacgaatgttagaaattatgtgcaccggattttggatgagcaaggagttttaatctacaagacttatggaacatatatttgtgagagcgaaaagaatgcagtaacaatccttggtcccatgttcaagacggtcgacttagttcaaacagaatttagtagttctcaaacgtctgaagtatatatggtatgtaaaggtttgaagaaattaatcgatgaacccaatcccgattggtcttccatcaatgaatcctggaaaaacctgtacgcattccagtcatcagaacaggaatttgccagagcaaagaaggttagtacatactttaccttgacaggtattccctcccaattcattcctgatccttttgtaaacattgagactatgctacaaatattcggagtacccacgggtgtgtctcatgcggctgccttaaaatcatctgatagacctgcagatttattgaccattagccttttttatatggcgattatatcgtattataacatcaatcatatcagagtaggaccgatacctccgaaccccccatcagatggaattgcacaaaatgtggggatcgctataactggtataagcttttggctgagtttgatggagaaagacattccactatatcaacagtgtttagcagttatccagcaatcattcccgattaggtgggaggctgtttcagtaaaaggaggatacaagcagaagtggagtactagaggtgatgggctcccaaaagatacccgaatttcagactccttggccccaatcgggaactggatcagatctctggaattggtccgaaaccaagttcgtctaaatccattcaatgagatcttgttcaatcagctatgtcgtacagtggataatcatttgaaatggtcaaatttgcgaagaaacacaggaatgattgaatggatcaatagacgaatttcaaaagaagaccggtctatactgatgttgaagagtgacctacacgaggaaaactcttggagagattaaaaaatcatgaggagactccaaactttaagtatgaaaaaaactttgatccttaagaccctcttgtggtttttattttttatctggttttgtggtcttcgtgggtcggcatggcatctccacctcctcgcggtccgacctgggcatccgaaggaggacgtcgtccactcggatggctaagggaggggcccccgcggggctgctaacaaagcccgaaaggaagctgagttggctgctgccaccgctgagcaataactagcataaccccttggggcctctaaacgggtcttgaggggttttttgctgaaaggaggaactatatccggatcgagacctcgatactagtgcggtggagctccagcttttgttccctttagtgagggttaattgcgcgcttggcgtaatcatggtcatagctgtttcctgtgtgaaattgttatccgctcacaattccacacaacatacgagccggaagcataaagtgtaaagcctggggtgcctaatgagtgagctaactcacattaattgcgttgcgctcactgcccgctttccagtcgggaaacctgtcgtgccagctgcattaatgaatcggccaacgcgcggggagaggcggtttgcgtattgggcgctcttccgcttcctcgctcactgactcgctgcgctcggtcgttcggctgcggcgagcggtatcagctcactcaaaggcggtaatacggttatccacagaatcaggggataacgcaggaaagaacatgtgagcaaaaggccagcaaaaggccaggaaccgtaaaaaggccgcgttgctggcgtttttccataggctccgcccccctgacgagcatcacaaaaatcgacgctcaagtcagaggtggcgaaacccgacaggactataaagataccaggcgtttccccctggaagctccctcgtgcgctctcctgttccgaccctgccgcttaccggatacctgtccgcctttctcccttcgggaagcgtggcgctttctcatagctcacgctgtaggtatctcagttcggtgtaggtcgttcgctccaagctgggctgtgtgcacgaaccccccgttcagcccgaccgctgcgccttatccggtaactatcgtcttgagtccaacccggtaagacacgacttatcgccactggcagcagccactggtaacaggattagcagagcgaggtatgtaggcggtgctacagagttcttgaagtggtggcctaactacggctacactagaaggacagtatttggtatctgcgctctgctgaagccagttaccttcggaaaaagagttggtagctcttgatccggcaaacaaaccaccgctggtagcggtggtttttttgtttgcaagcagcagattacgcgcagaaaaaaaggatctcaagaagatcctttgatcttttctacggggtctgacgctcagtggaacgaaaactcacgttaagggattttggtcatgagattatcaaaaaggatcttcacctagatccttttaaattaaaaatgaagttttaaatcaatctaaagtatatatgagtaaacttggtctgacagttaccaatgcttaatcagtgaggcacctatctcagcgatctgtctatttcgttcatccatagttgcctgactccccgtcgtgtagataactacgatacgggagggcttaccatctggccccagtgctgcaatgataccgcgagacccacgctcaccggctccagatttatcagcaataaaccagccagccggaagggccgagcgcagaagtggtcctgcaactttatccgcctccatccagtctattaattgttgccgggaagctagagtaagtagttcgccagttaatagtttgcgcaacgttgttgccattgctacaggcatcgtggtgtcacgctcgtcgtttggtatggcttcattcagctccggttcccaacgatcaaggcgagttacatgatcccccatgttgtgcaaaaaagcggttagctccttcggtcctccgatcgttgtcagaagtaagttggccgcagtgttatcactcatggttatggcagcactgcataattctcttactgtcatgccatccgtaagatgcttttctgtgactggtgagtactcaaccaagtcattctgagaatagtgtatgcggcgaccgagttgctcttgcccggcgtcaatacgggataataccgcgccacatagcagaactttaaaagtgctcatcattggaaaacgttcttcggggcgaaaactctcaaggatcttaccgctgttgagatccagttcgatgtaacccactcgtgcacccaactgatcttcagcatcttttactttcaccagcgtttctgggtgagcaaaaacaggaaggcaaaatgccgcaaaaaagggaataagggcgacacggaaatgttgaatactcatactcttcctttttcaatattattgaagcatttatcagggttattgtctcatgagcggatacatatttgaatgtatttagaaaaataaacaaataggggttccgcgcacatttccccgaaaagtgccac

SEQ ID NO: 14 - RNA, 14579 nt, synthetic construct
  source 1..14579: mol_type = other RNA
ctaaattgtaagcgttaatattttgttaaaattcgcgttaaatttttgttaaatcagctcattttttaaccaataggccgaaatcggcaaaatcccttataaatcaaaagaatagaccgagatagggttgagtgttgttccagtttggaacaagagtccactattaaagaacgtggactccaacgtcaaagggcgaaaaaccgtctatcagggcgatggcccactacgtgaaccatcaccctaatcaagttttttggggtcgaggtgccgtaaagcactaaatcggaaccctaaagggagcccccgatttagagcttgacggggaaagccggcgaacgtggcgagaaaggaagggaagaaagcgaaaggagcgggcgctagggcgctggcaagtgtagcggtcacgctgcgcgtaaccaccacacccgccgcgcttaatgcgccgctacagggcgcgtcccattcgccattcaggctgcgcaactgttgggaagggcgatcggtgcgggcctcttcgctattacgccagctggcgaaagggggatgtgctgcaaggcgattaagttgggtaacgccagggttttcccagtcacgacgttgtaaaacgacggccagtgagcgcgcgtaatacgactcactatagggacgaagacaaacaaaccattattatcattaaaaggctcaggagaaactttaacagtaatcaaaatgtctgttacagtcaagagaatcattgacaacacagtcgtagttccaaaacttcctgcaaatgaggatccagtggaatacccggcagattacttcagaaaatcaaaggagattcctctttacatcaatactacaaaaagtttgtcagatctaagaggatatgtctaccaaggcctcaaatccggaaatgtatcaatcatacatgtcaacagctacttgtatggagcattaaaggacatccggggtaagttggataaagattggtcaagtttcggaataaacatcgggaaagcaggggatacaatcggaatatttgaccttgtatccttgaaagccctggacggcgtacttccagatggagtatcggatgcttccagaaccagcgcagatgacaaatggttgcctttgtatctacttggcttatacagagtgggcagaacacaaatgcctgaatacagaaaaaagctcatggatgggctgacaaatcaatgcaaaatgatcaatgaacagtttgaacctcttgtgccagaaggtcgtgacatttttgatgtgtggggaaatgacagtaattacacaaaaattgtcgctgcagtggacatgttcttccacatgttcaaaaaacatgaatgtgcctcgttcagatacggaactattgtttccagattcaaagattgtgctgcattggcaacatttggacacctctgcaaaataaccggaatgtctacagaagatgtaacgacctggatcttgaaccgagaagttgcagatgaaatggtccaaatgatgcttccaggccaagaaattgacaaggccgattcatacatgccttatttgatcgactttggattgtcttctaagtctccatattcttccgtcaaaaaccctgccttccacttctgggggcaattgacagctcttctgctcagatccaccagagcaaggaatgcccgacagcctgatgacattgagtatacatctcttactacagcaggtttgttgtacgcttatgcagtaggatcctctgccgacttggcacaacagttttgtgttggagataacaaatacactccagatgatagtaccggaggattgacgactaatgcaccgccacaaggcagagatgtggtcgaatggctcggatggtttgaagatcaaaacagaaaaccgactcctgatatgatgcagtatgcgaaaagagcagtcatgtcactgcaaggcctaagagagaagacaattggcaagtatgctaagtcagaatttgacaaatgaccctataattctcagatcacctattatatattatgctacatatgaaaaaaactaacagatatcatggataatctcacaaaagttcgtgagtatctcaagtcctattctcgtctggatcaggcggtaggagagatagatgagatcgaagcacaacgagctgaaaagtccaattatgagttgttccaagaggatggagtggaagagcatactaagccctcttattttcaggcagcagatgattctgacacagaatctgaaccagaaattgaagacaatcaaggcttgtatgcaccagatccagaagctgagcaagttgaaggctttatacaggggcctttagatgactatgcagatgaggaagtggatgttgtatttacttcggactggaaacagcctgagcttgaatctgacgagcatggaaagaccttacggttgacatcgccagagggtttaagtggagagcagaaatcccagtggctttcgacgattaaagcagtcgtgcaaagtgccaaatactggaatctggcagagtgcacatttgaagcatcgggagaaggggtcattatgaaggagcgccagataactccggatgtatataaggtcactccagtgatgaacacacatccgtcccaatcagaagcagtatcagatgtttggtctctctcaaagacatccatgactttccaacccaagaaagcaagtcttcagcctctcaccatatccttggatgaattgttctcatctagaggagagttcatctctgtcggaggtgacggacgaatgtctcataaagaggccatcctgctcggcctgagatacaaaaagttgtacaatcaggcgagagtcaaatattctctgtagactatgaaaaaaagtaacagatatcacgatctaagtgttatcccaatccattcatcatgagttccttaaagaagattctcggtctgaaggggaaaggtaagaaatctaagaaattagggatcgcaccacccccttatgaagaggacactagcatggagtatgctccgagcgctccaattgacaaatcctattttggagttgacgagatggacacctatgatccgaatcaattaagatatgagaaattcttctttacagtgaaaatgacggttagatctaatcgtccgttcagaacatactcagatgtggcagccgctgtatcccattgggatcacatgtacatcggaatggcagggaaacgtcccttctacaaaatcttggcttttttgggttcttctaatctaaaggccactccagcggtattggcagatcaaggtcaaccagagtatcacgctcactgcgaaggcagggcttatttgccacataggatggggaagacccctcccatgctcaatgtaccagagcacttcagaagaccattcaatataggtctttacaagggaacgattgagctcacaatgaccatctacgatgatgagtcactggaagcagctcctatgatctgggatcatttcaattcttccaaattttctgatttcagagagaaggccttaatgtttggcctgattgtcgagaaaaaggcatctggagcgtgggtcctggactctatcggccacttcaaatgagctagtctaacttctagcttctgaacaatccccggtttactcagtctcccctaattccagcctctcgaacaactaatatcctgtcttttctatccctatgaaaaaaactaacagagatcgatctgtttacgcgtaaaatggacctcatggggtacatccctgtcgtgggcgccccgctcggcggcgtcgccagagctctcgcgcatggcgtgagagtcctggaggacggggttaattttgcaacagggaacttacccggttgctccttttctatcttcttgctggccctgctgtcctgcatcaccaccccggtctccgctgtgcaagtcaagaacaccagcacaatgtaccaggtgactaatgactgtcctaactccagtatagtctggcagcttaaggatgccgtccttcacgtccctgggtgtgtcccctgtgagcaagtgaacaacatgtcccggtgttggttaccggtcactcccaatgtggccatcagccaacctggggccctcactaggggcttgcggacgcacattgacattattgtgatgtccgccactctgtgctcagccctctatgtgggggatgtgtgtggcggggtgatgatagcctctcaggctttcgttgtctcgccgcaaatgcaccacttcgtccaggactgcaactgttccatctatccgggccatgtcacgggacatcgtatggcatgggatatgatgatgaattggtcgccgactgccaccatgatcatggcatatgcggtgcgtatccccgagcttgccttggagatcatcgctggcggccattggggtgtgctgtttggcctagcttacttctccttgcaaggagcgtgggcgaaggtcgtcgtcatcctcctgctgtttgcaggagtggaggcgcatacccacgtagttgggggcagcgtagcccagggcgcccggggctttactggcctgttctccccggggtcccagcagaacattcagcttattaacaccaatggtagttggcacattaaccgcacggccctcaattgcaatgatagccttaacaccggcttccttgcttctctgttctacacccataagttcaactcctcaggctgtccggagcgcatgtctgcctgtaagggcattgaggcgttccggatagggtggggtgtcttggaacatgaggagaacgtgaccaacgatgaggacatgaggccctactgctggcactacccgcctaaaccttgtggtatcgttccagctcgaacggtatgtggcccagtctactgcttcacccccagtccagtagtagtgggcactaccgacaggcgcggtgtgcccacttacacctggggggaaaatgagacagatgtctttctgctcaacagcacccgcccccctgggggcagttggtttgggtgcacgtggatgaactccactggctacaccaagacctgcggcgcaccaccttgccgcatcagagcagatttcaatgccagcacagacctactatgccccacagactgctttaggaagcatcccgatgcgacctatggcaagtgtggggctggaccctggttaactccaaaatgtctggttgactacccctacaggctgtggcactacccgtgcacagtcaatttcaccatctttaagatcaggatgtacgtggggggagtcgaacacaggctacaagcagcgtgtaacttcagtcgtggagaccgctgtaatctggaggacagggataggagccaattaagcccacttctgcattccaccactgagtgggccatcctaccctgcactttttcagatatgccggctttgtcaacagggttgctgcatcttcaccagaatatcgtggacgtgcagtacttgtatggtctgtcaccggccctcacaaaatacatggtcaaatgggaatgggtggtcctgctcttcctgctcttagcagatgctaggatctgcgcatgtctttggatgctcatcctgatgggccaggctgaggcataagctagccagattcttcatgtttggaccaaatcaacttgtgataccatgctcaaagaggcctcaattatatttgagtttttaatttttatgaaaaaaactaacagcaatcatggaagtccacgattttgagaccgacgagttcaatgatttcaatgaagatgactatgccacaagagaattcctgaatcccgatgagcgcatgacgtacttgaatcatgctgattacaacctgaattctcctctaattagtgatgatattgacaatttaatcaggaaattcaattctcttccaattccctcgatgtgggatagtaagaactgggatggagttcttgagatgttaacgtcatgtcaagccaatcccatcccaacatctcagatgcataaatggatgggaagttggttaatgtctgataatcatgatgccagtcaagggtatagttttttacatgaagtggacaaagaggcagaaataacatttgacgtggtggagaccttcatccgcggctggggcaacaaaccaattgaatacatcaaaaaggaaagatggactgactcattcaaaattctcgcttatttgtgtcaaaagtttttggacttacacaagttgacattaatcttaaatgctgtctctgaggtggaattgctcaacttggcgaggactttcaaaggcaaagtcagaagaagttctcatggaacgaacatatgcaggattagggttcccagcttgggtcctacttttatttcagaaggatgggcttacttcaagaaacttgatattctaatggaccgaaactttctgttaatggtcaaagatgtgattatagggaggatgcaaacggtgctatccatggtatgtagaatagacaacctgttctcagagcaagacatcttctcccttctaaatatctacagaattggagataaaattgtggagaggcagggaaatttttcttatgacttgattaaaatggtggaaccgatatgcaacttgaagctgatgaaattagcaagagaatcaaggcctttagtcccacaattccctcattttgaaaatcatatcaagacttctgttgatgaaggggcaaaaattgaccgaggtataagattcctccatgatcagataatgagtgtgaaaacagtggatctcacactggtgatttatggatcgttcagacattggggtcatccttttatagattattacactggactagaaaaattacattcccaagtaaccatgaagaaagatattgatgtgtcatatgcaaaagcacttgcaagtgatttagctcggattgttctatttcaacagttcaatgatcataaaaagtggttcgtgaatggagacttgctccctcatgatcatccctttaaaagtcatgttaaagaaaatacatggcccacagctgctcaagttcaagattttggagataaatggcatgaacttccgctgattaaatgttttgaaatacccgacttactagacccatcgataatatactctgacaaaagtcattcaatgaataggtcagaggtgttgaaacatgtccgaatgaatccgaacactcctatccctagtaaaaaggtgttgcagactatgttggacacaaaggctaccaattggaaagaatttcttaaagagattgatgagaagggcttagatgatgatgatctaattattggtcttaaaggaaaggagagggaactgaagttggcaggtagatttttctccctaatgtcttggaaattgcgagaatactttgtaattaccgaatatttgataaagactcatttcgtccctatgtttaaaggcctgacaatggcggacgatctaactgcagtcattaaaaagatgttagattcctcatccggccaaggattgaagtcatatgaggcaatttgcatagccaatcacattgattacgaaaaatggaataaccaccaaaggaagttatcaaacggcccagtgttccgagttatgggccagttcttaggttatccatccttaatcgagagaactcatgaattttttgagaaaagtcttatatactacaatggaagaccagacttgatgcgtgttcacaacaacacactgatcaattcaacctcccaacgagtttgttggcaaggacaagagggtggactggaaggtctacggcaaaaaggatggagtatcctcaatctactggttattcaaagagaggctaaaatcagaaacactgctgtcaaagtcttggcacaaggtgataatcaagttatttgcacacagtataaaacgaagaaatcgagaaacgttgtagaattacagggtgctctcaatcaaatggtttctaataatgagaaaattatgactgcaatcaaaatagggacagggaagttaggacttttgataaatgacgatgagactatgcaatctgcagattacttgaattatggaaaaataccgattttccgtggagtgattagagggttagagaccaagagatggtcacgagtgacttgtgtcaccaatgaccaaatacccacttgtgctaatataatgagctcagtttccacaaatgctctcaccgtagctcattttgctgagaacccaatcaatgccatgatacagtacaattattttgggacatttgctagactcttgttgatgatgcatgatcctgctcttcgtcaatcattgtatgaagttcaagataagataccgggcttgcacagttctactttcaaatacgccatgttgtatttggacccttccattggaggagtgtcgggcatgtctttgtccaggtttttgattagagccttcccagatcccgtaacagaaagtctctcattctggagattcatccatgtacatgctcgaagtgagcatctgaaggagatgagtgcagtatttggaaaccccgagatagccaagtttcgaataactcacatagacaagctagtagaagatccaacctctctgaacatcgctatgggaatgagtccagcgaacttgttaaagactgaggttaaaaaatgcttaatcgaatcaagacaaaccatcaggaaccaggtgattaaggatgcaaccatatatttgtatcatgaagaggatcggctcagaagtttcttatggtcaataaatcctctgttccctagatttttaagtgaattcaaatcaggcacttttttgggagtcgcagacgggctcatcagtctatttcaaaattctcgtactattcggaactcctttaagaaaaagtatcatagggaattggatgatttgattgtgaggagtgaggtatcctctttgacacatttagggaaacttcatttgagaaggggatcatgtaaaatgtggacatgttcagctactcatgctgacacattaagatacaaatcctggggccgtacagttattgggacaactgtaccccatccattagaaatgttgggtccacaacatcgaaaagagactccttgtgcaccatgtaacacatcagggttcaattatgtttctgtgcattgtccagacgggatccatgacgtctttagttcacggggaccattgcctgcttatctagggtctaaaacatctgaatctacatctattttgcagccttgggaaagggaaagcaaagtcccactgattaaaagagctacacgtcttagagatgctatctcttggtttgttgaacccgactctaaactagcaatgactatactttctaacatccactctttaacaggcgaagaatggaccaaaaggcagcatgggttcaaaagaacagggtctgcccttcataggttttcgacatctcggatgagccatggtgggttcgcatctcagagcactgcagcattgaccaggttgatggcaactacagacaccatgagggatctgggagatcagaatttcgactttttattccaagcaacgttgctctatgctcaaattaccaccactgttgcaagagacggatggatcaccagttgtacagatcattatcatattgcctgtaagtcctgtttgagacccatagaagagatcaccctggactcaagtatggactacacgcccccagatgtatcccatgtgctgaagacatggaggaatggggaaggttcgtggggacaagagataaaacagatctatcctttagaagggaattggaagaatttagcacctgctgagcaatcctatcaagtcggcagatgtataggttttctatatggagacttggcgtatagaaaatctactcatgccgaggacagttctctatttcctctatctatacaaggtcgtattagaggtcgaggtttcttaaaagggttgctagacggattaatgagagcaagttgctgccaagtaatacaccggagaagtctggctcatttgaagaggccggccaacgcagtgtacggaggtttgatttacttgattgataaattgagtgtatcacctccattcctttctcttactagatcaggacctattagagacgaattagaaacgattccccacaagatcccaacctcctatccgacaagcaaccgtgatatgggggtgattgtcagaaattacttcaaataccaatgccgtctaattgaaaagggaaaatacagatcacattattcacaattatggttattctcagatgtcttatccatagacttcattggaccattctctatttccaccaccctcttgcaaatcctatacaagccatttttatctgggaaagataagaatgagttgagagagctggcaaatctttcttcattgctaagatcaggagaggggtgggaagacatacatgtgaaattcttcaccaaggacatattattgtgtccagaggaaatcagacatgcttgcaagttcgggattgctaaggataataataaagacatgagctatcccccttggggaagggaatccagagggacaattacaacaatccctgtttattatacgaccaccccttacccaaagatgctagagatgcctccaagaatccaaaatcccctgctgtccggaatcaggttgggccaattaccaactggcgctcattataaaattcggagtatattacatggaatgggaatccattacagggacttcttgagttgtggagacggctccggagggatgactgctgcattactacgagaaaatgtgcatagcagaggaatattcaatagtctgttagaattatcagggtcagtcatgcgaggcgcctctcctgagccccccagtgccctagaaactttaggaggagataaatcgagatgtgtaaatggtgaaacatgttgggaatatccatctgacttatgtgacccaaggacttgggactatttcctccgactcaaagcaggcttggggcttcaaattgatttaattgtaatggatatggaagttcgggattcttctactagcctgaaaattgagacgaatgttagaaattatgtgcaccggattttggatgagcaaggagttttaatctacaagacttatggaacatatatttgtgagagcgaaaagaatgcagtaacaatccttggtcccatgttcaagacggtcgacttagttcaaacagaatttagtagttctcaaacgtctgaagtatatatggtatgtaaaggtttgaagaaattaatcgatgaacccaatcccgattggtcttccatcaatgaatcctggaaaaacctgtacgcattccagtcatcagaacaggaatttgccagagcaaagaaggttagtacatactttaccttgacaggtattccctcccaattcattcctgatccttttgtaaacattgagactatgctacaaatattcggagtacccacgggtgtgtctcatgcggctgccttaaaatcatctgatagacctgcagatttattgaccattagccttttttatatggcgattatatcgtattataacatcaatcatatcagagtaggaccgatacctccgaaccccccatcagatggaattgcacaaaatgtggggatcgctataactggtataagcttttggctgagtttgatggagaaagacattccactatatcaacagtgtttagcagttatccagcaatcattcccgattaggtgggaggctgtttcagtaaaaggaggatacaagcagaagtggagtactagaggtgatgggctcccaaaagatacccgaatttcagactccttggccccaatcgggaactggatcagatctctggaattggtccgaaaccaagttcgtctaaatccattcaatgagatcttgttcaatcagctatgtcgtacagtggataatcatttgaaatggtcaaatttgcgaagaaacacaggaatgattgaatggatcaatagacgaatttcaaaagaagaccggtctatactgatgttgaagagtgacctacacgaggaaaactcttggagagattaaaaaatcatgaggagactccaaactttaagtatgaaaaaaactttgatccttaagaccctcttgtggtttttattttttatctggttttgtggtcttcgtgggtcggcatggcatctccacctcctcgcggtccgacctgggcatccgaaggaggacgtcgtccactcggatggctaagggaggggcccccgcggggctgctaacaaagcccgaaaggaagctgagttggctgctgccaccgctgagcaataactagcataaccccttggggcctctaaacgggtcttgaggggttttttgctgaaaggaggaactatatccggatcgagacctcgatactagtgcggtggagctccagcttttgttccctttagtgagggttaattgcgcgcttggcgtaatcatggtcatagctgtttcctgtgtgaaattgttatccgctcacaattccacacaacatacgagccggaagcataaagtgtaaagcctggggtgcctaatgagtgagctaactcacattaattgcgttgcgctcactgcccgctttccagtcgggaaacctgtcgtgccagctgcattaatgaatcggccaacgcgcggggagaggcggtttgcgtattgggcgctcttccgcttcctcgctcactgactcgctgcgctcggtcgttcggctgcggcgagcggtatcagctcactcaaaggcggtaatacggttatccacagaatcaggggataacgcaggaaagaacatgtgagcaaaaggccagcaaaaggccaggaaccgtaaaaaggccgcgttgctggcgtttttccataggctccgcccccctgacgagcatcacaaaaatcgacgctcaagtcagaggtggcgaaacccgacaggactataaagataccaggcgtttccccctggaagctccctcgtgcgctctcctgttccgaccctgccgcttaccggatacctgtccgcctttctcccttcgggaagcgtggcgctttctcatagctcacgctgtaggtatctcagttcggtgtaggtcgttcgctccaagctgggctgtgtgcacgaaccccccgttcagcccgaccgctgcgccttatccggtaactatcgtcttgagtccaacccggtaagacacgacttatcgccactggcagcagccactggtaacaggattagcagagcgaggtatgtaggcggtgctacagagttcttgaagtggtggcctaactacggctacactagaaggacagtatttggtatctgcgctctgctgaagccagttaccttcggaaaaagagttggtagctcttgatccggcaaacaaaccaccgctggtagcggtggtttttttgtttgcaagcagcagattacgcgcagaaaaaaaggatctcaagaagatcctttgatcttttctacggggtctgacgctcagtggaacgaaaactcacgttaagggattttggtcatgagattatcaaaaaggatcttcacctagatccttttaaattaaaaatgaagttttaaatcaatctaaagtatatatgagtaaacttggtctgacagttaccaatgcttaatcagtgaggcacctatctcagcgatctgtctatttcgttcatccatagttgcctgactccccgtcgtgtagataactacgatacgggagggcttaccatctggccccagtgctgcaatgataccgcgagacccacgctcaccggctccagatttatcagcaataaaccagccagccggaagggccgagcgcagaagtggtcctgcaactttatccgcctccatccagtctattaattgttgccgggaagctagagtaagtagttcgccagttaatagtttgcgcaacgttgttgccattgctacaggcatcgtggtgtcacgctcgtcgtttggtatggcttcattcagctccggttcccaacgatcaaggcgagttacatgatcccccatgttgtgcaaaaaagcggttagctccttcggtcctccgatcgttgtcagaagtaagttggccgcagtgttatcactcatggttatggcagcactgcataattctcttactgtcatgccatccgtaagatgcttttctgtgactggtgagtactcaaccaagtcattctgagaatagtgtatgcggcgaccgagttgctcttgcccggcgtcaatacgggataataccgcgccacatagcagaactttaaaagtgctcatcattggaaaacgttcttcggggcgaaaactctcaaggatcttaccgctgttgagatccagttcgatgtaacccactcgtgcacccaactgatcttcagcatcttttactttcaccagcgtttctgggtgagcaaaaacaggaaggcaaaatgccgcaaaaaagggaataagggcgacacggaaatgttgaatactcatactcttcctttttcaatattattgaagcatttatcagggttattgtctcatgagcggatacatatttgaatgtatttagaaaaataaacaaataggggttccgcgcacatttccccgaaaagtgccac

SEQ ID NO: 15 - RNA, 14570 nt, synthetic construct
  source 1..14570: mol_type = other RNA
ctaaattgtaagcgttaatattttgttaaaattcgcgttaaatttttgttaaatcagctcattttttaaccaataggccgaaatcggcaaaatcccttataaatcaaaagaatagaccgagatagggttgagtgttgttccagtttggaacaagagtccactattaaagaacgtggactccaacgtcaaagggcgaaaaaccgtctatcagggcgatggcccactacgtgaaccatcaccctaatcaagttttttggggtcgaggtgccgtaaagcactaaatcggaaccctaaagggagcccccgatttagagcttgacggggaaagccggcgaacgtggcgagaaaggaagggaagaaagcgaaaggagcgggcgctagggcgctggcaagtgtagcggtcacgctgcgcgtaaccaccacacccgccgcgcttaatgcgccgctacagggcgcgtcccattcgccattcaggctgcgcaactgttgggaagggcgatcggtgcgggcctcttcgctattacgccagctggcgaaagggggatgtgctgcaaggcgattaagttgggtaacgccagggttttcccagtcacgacgttgtaaaacgacggccagtgagcgcgcgtaatacgactcactatagggacgaagacaaacaaaccattattatcattaaaaggctcaggagaaactttaacagtaatcaaaatgtctgttacagtcaagagaatcattgacaacacagtcgtagttccaaaacttcctgcaaatgaggatccagtggaatacccggcagattacttcagaaaatcaaaggagattcctctttacatcaatactacaaaaagtttgtcagatctaagaggatatgtctaccaaggcctcaaatccggaaatgtatcaatcatacatgtcaacagctacttgtatggagcattaaaggacatccggggtaagttggataaagattggtcaagtttcggaataaacatcgggaaagcaggggatacaatcggaatatttgaccttgtatccttgaaagccctggacggcgtacttccagatggagtatcggatgcttccagaaccagcgcagatgacaaatggttgcctttgtatctacttggcttatacagagtgggcagaacacaaatgcctgaatacagaaaaaagctcatggatgggctgacaaatcaatgcaaaatgatcaatgaacagtttgaacctcttgtgccagaaggtcgtgacatttttgatgtgtggggaaatgacagtaattacacaaaaattgtcgctgcagtggacatgttcttccacatgttcaaaaaacatgaatgtgcctcgttcagatacggaactattgtttccagattcaaagattgtgctgcattggcaacatttggacacctctgcaaaataaccggaatgtctacagaagatgtaacgacctggatcttgaaccgagaagttgcagatgaaatggtccaaatgatgcttccaggccaagaaattgacaaggccgattcatacatgccttatttgatcgactttggattgtcttctaagtctccatattcttccgtcaaaaaccctgccttccacttctgggggcaattgacagctcttctgctcagatccaccagagcaaggaatgcccgacagcctgatgacattgagtatacatctcttactacagcaggtttgttgtacgcttatgcagtaggatcctctgccgacttggcacaacagttttgtgttggagataacaaatacactccagatgatagtaccggaggattgacgactaatgcaccgccacaaggcagagatgtggtcgaatggctcggatggtttgaagatcaaaacagaaaaccgactcctgatatgatgcagtatgcgaaaagagcagtcatgtcactgcaaggcctaagagagaagacaattggcaagtatgctaagtcagaatttgacaaatgaccctataattctcagatcacctattatatattatgctacatatgaaaaaaactaacagatatcatggataatctcacaaaagttcgtgagtatctcaagtcctattctcgtctggatcaggcggtaggagagatagatgagatcgaagcacaacgagctgaaaagtccaattatgagttgttccaagaggatggagtggaagagcatactaagccctcttattttcaggcagcagatgattctgacacagaatctgaaccagaaattgaagacaatcaaggcttgtatgcaccagatccagaagctgagcaagttgaaggctttatacaggggcctttagatgactatgcagatgaggaagtggatgttgtatttacttcggactggaaacagcctgagcttgaatctgacgagcatggaaagaccttacggttgacatcgccagagggtttaagtggagagcagaaatcccagtggctttcgacgattaaagcagtcgtgcaaagtgccaaatactggaatctggcagagtgcacatttgaagcatcgggagaaggggtcattatgaaggagcgccagataactccggatgtatataaggtcactccagtgatgaacacacatccgtcccaatcagaagcagtatcagatgtttggtctctctcaaagacatccatgactttccaacccaagaaagcaagtcttcagcctctcaccatatccttggatgaattgttctcatctagaggagagttcatctctgtcggaggtgacggacgaatgtctcataaagaggccatcctgctcggcctgagatacaaaaagttgtacaatcaggcgagagtcaaatattctctgtagactatgaaaaaaagtaacagatatcacgatctaagtgttatcccaatccattcatcatgagttccttaaagaagattctcggtctgaaggggaaaggtaagaaatctaagaaattagggatcgcaccacccccttatgaagaggacactagcatggagtatgctccgagcgctccaattgacaaatcctattttggagttgacgagatggacacctatgatccgaatcaattaagatatgagaaattcttctttacagtgaaaatgacggttagatctaatcgtccgttcagaacatactcagatgtggcagccgctgtatcccattgggatcacatgtacatcggaatggcagggaaacgtcccttctacaaaatcttggcttttttgggttcttctaatctaaaggccactccagcggtattggcagatcaaggtcaaccagagtatcacgctcactgcgaaggcagggcttatttgccacataggatggggaagacccctcccatgctcaatgtaccagagcacttcagaagaccattcaatataggtctttacaagggaacgattgagctcacaatgaccatctacgatgatgagtcactggaagcagctcctatgatctgggatcatttcaattcttccaaattttctgatttcagagagaaggccttaatgtttggcctgattgtcgagaaaaaggcatctggagcgtgggtcctggactctatcggccacttcaaatgagctagtctaacttctagcttctgaacaatccccggtttactcagtctcccctaattccagcctctcgaacaactaatatcctgtcttttctatccctatgaaaaaaactaacagagatcgatctgtttacgcgtaaaatggacctcatggggtacatcccgctcgtaggcggccccgttgggggcgtcgcaagggctctcgcacacggtgtgagggtccttgaggacggggtaaactatgcaacagggaatttacccggttgctctttctctatctttatccttgcacttctttcatgcctgactgtcccgacctctgccgttccctaccgaaatgcctctggggtttatcatgtcaccaatgattgcccaaactcttctatcgtctatgaggctgaagacctgatcttacacgcacctggttgcgtgccctgtgttaggcagggtaatgtcagtaggtgctgggtccagatcacccccacactgtcagccccgagcctcggagcggtcacggctcctcttcggagggccgttgactacttagcggggggggctgccctttgctccgcgttatacgtcggagacgcgtgcggggcagtgtttttggtaggtcaaatgttcacctatagccctcgccggcataatgttgtgcaggactgcaactgttccatttacagtggccacatcaccggccaccggatggcatgggacatgatgatgaattggtcacctacaacagctttggtgatggcccagttgttacggattccccaggtggtcattgacatcattgccggggcccactggggggtcttgttcgccgccgcatactacgcgtcggcggctaactgggccaaggttgtgctggtcctgtttctgtttgcgggggtcgatgccagcacccgcactgtgggtggtagtgcggcccaaggcgcgcgcgggctcgcttcacttttcacccctgggccgcagcagaacttgcagctcataaataccaacgggagctggcacatcaacagaactgcccttaactgtaatgacagcctccagactgggtttgtagccggcctcctgtattatcacaagttcaactccactgggtgtccgcagcggatggctagctgtaggcccctcgccgcattcgaccagggctggggaactatcagctatgccgccgtgtcgggccccagtgatgacaagccctattgctggcactaccccccacgcccgtgcggaatagtgccagcgcgaggtgtctgcggtccggtctattgttttacacctagcccggtggtcgtcggcaccacagaccgcaaggggaatcccacttacagttggggcgaaaatgagactgacatctttctcttgaacaacacgaggccccctactggcaactggtttggctgcacctggatgaattccacagggtttgtcaagacttgcggggctccaccctgcaacttagggcctacaggcaacaatagccttaagtgtcctactgattgcttccgcaagcacccagacgccacctacaccaagtgtgggtcaggaccctggctcactccccggtgtctggtgcattacccttaccggttgtggcattacccgtgcaccctaaattacaccatcttcaaggtgcgcatgtacattgggggcctcgagcacaggctcgaggtggcatgcaactggacccgtggtgagcggtgtgatcttgaagacagggatagggccgagctgagcccgctcctacataccaccacgcagtgggccatattgccgtgctctttcacacccacacccgctcttagcactggtctcatacacttacatcaaaatatagtagacacccagtatctttacggtctgagctccagcatcgtctcgtgggccgttaagtgggagtacatagtgctggccttcttattacttgctgatgcccgtatttgtacttgcctatggatcatgctcctggtttgtcaggccgaagcgtaagctagccagattcttcatgtttggaccaaatcaacttgtgataccatgctcaaagaggcctcaattatatttgagtttttaatttttatgaaaaaaactaacagcaatcatggaagtccacgattttgagaccgacgagttcaatgatttcaatgaagatgactatgccacaagagaattcctgaatcccgatgagcgcatgacgtacttgaatcatgctgattacaacctgaattctcctctaattagtgatgatattgacaatttaatcaggaaattcaattctcttccaattccctcgatgtgggatagtaagaactgggatggagttcttgagatgttaacgtcatgtcaagccaatcccatcccaacatctcagatgcataaatggatgggaagttggttaatgtctgataatcatgatgccagtcaagggtatagttttttacatgaagtggacaaagaggcagaaataacatttgacgtggtggagaccttcatccgcggctggggcaacaaaccaattgaatacatcaaaaaggaaagatggactgactcattcaaaattctcgcttatttgtgtcaaaagtttttggacttacacaagttgacattaatcttaaatgctgtctctgaggtggaattgctcaacttggcgaggactttcaaaggcaaagtcagaagaagttctcatggaacgaacatatgcaggattagggttcccagcttgggtcctacttttatttcagaaggatgggcttacttcaagaaacttgatattctaatggaccgaaactttctgttaatggtcaaagatgtgattatagggaggatgcaaacggtgctatccatggtatgtagaatagacaacctgttctcagagcaagacatcttctcccttctaaatatctacagaattggagataaaattgtggagaggcagggaaatttttcttatgacttgattaaaatggtggaaccgatatgcaacttgaagctgatgaaattagcaagagaatcaaggcctttagtcccacaattccctcattttgaaaatcatatcaagacttctgttgatgaaggggcaaaaattgaccgaggtataagattcctccatgatcagataatgagtgtgaaaacagtggatctcacactggtgatttatggatcgttcagacattggggtcatccttttatagattattacactggactagaaaaattacattcccaagtaaccatgaagaaagatattgatgtgtcatatgcaaaagcacttgcaagtgatttagctcggattgttctatttcaacagttcaatgatcataaaaagtggttcgtgaatggagacttgctccctcatgatcatccctttaaaagtcatgttaaagaaaatacatggcccacagctgctcaagttcaagattttggagataaatggcatgaacttccgctgattaaatgttttgaaatacccgacttactagacccatcgataatatactctgacaaaagtcattcaatgaataggtcagaggtgttgaaacatgtccgaatgaatccgaacactcctatccctagtaaaaaggtgttgcagactatgttggacacaaaggctaccaattggaaagaatttcttaaagagattgatgagaagggcttagatgatgatgatctaattattggtcttaaaggaaaggagagggaactgaagttggcaggtagatttttctccctaatgtcttggaaattgcgagaatactttgtaattaccgaatatttgataaagactcatttcgtccctatgtttaaaggcctgacaatggcggacgatctaactgcagtcattaaaaagatgttagattcctcatccggccaaggattgaagtcatatgaggcaatttgcatagccaatcacattgattacgaaaaatggaataaccaccaaaggaagttatcaaacggcccagtgttccgagttatgggccagttcttaggttatccatccttaatcgagagaactcatgaattttttgagaaaagtcttatatactacaatggaagaccagacttgatgcgtgttcacaacaacacactgatcaattcaacctcccaacgagtttgttggcaaggacaagagggtggactggaaggtctacggcaaaaaggatggagtatcctcaatctactggttattcaaagagaggctaaaatcagaaacactgctgtcaaagtcttggcacaaggtgataatcaagttatttgcacacagtataaaacgaagaaatcgagaaacgttgtagaattacagggtgctctcaatcaaatggtttctaataatgagaaaattatgactgcaatcaaaatagggacagggaagttaggacttttgataaatgacgatgagactatgcaatctgcagattacttgaattatggaaaaataccgattttccgtggagtgattagagggttagagaccaagagatggtcacgagtgacttgtgtcaccaatgaccaaatacccacttgtgctaatataatgagctcagtttccacaaatgctctcaccgtagctcattttgctgagaacccaatcaatgccatgatacagtacaattattttgggacatttgctagactcttgttgatgatgcatgatcctgctcttcgtcaatcattgtatgaagttcaagataagataccgggcttgcacagttctactttcaaatacgccatgttgtatttggacccttccattggaggagtgtcgggcatgtctttgtccaggtttttgattagagccttcccagatcccgtaacagaaagtctctcattctggagattcatccatgtacatgctcgaagtgagcatctgaaggagatgagtgcagtatttggaaaccccgagatagccaagtttcgaataactcacatagacaagctagtagaagatccaacctctctgaacatcgctatgggaatgagtccagcgaacttgttaaagactgaggttaaaaaatgcttaatcgaatcaagacaaaccatcaggaaccaggtgattaaggatgcaaccatatatttgtatcatgaagaggatcggctcagaagtttcttatggtcaataaatcctctgttccctagatttttaagtgaattcaaatcaggcacttttttgggagtcgcagacgggctcatcagtctatttcaaaattctcgtactattcggaactcctttaagaaaaagtatcatagggaattggatgatttgattgtgaggagtgaggtatcctctttgacacatttagggaaacttcatttgagaaggggatcatgtaaaatgtggacatgttcagctactcatgctgacacattaagatacaaatcctggggccgtacagttattgggacaactgtaccccatccattagaaatgttgggtccacaacatcgaaaagagactccttgtgcaccatgtaacacatcagggttcaattatgtttctgtgcattgtccagacgggatccatgacgtctttagttcacggggaccattgcctgcttatctagggtctaaaacatctgaatctacatctattttgcagccttgggaaagggaaagcaaagtcccactgattaaaagagctacacgtcttagagatgctatctcttggtttgttgaacccgactctaaactagcaatgactatactttctaacatccactctttaacaggcgaagaatggaccaaaaggcagcatgggttcaaaagaacagggtctgcccttcataggttttcgacatctcggatgagccatggtgggttcgcatctcagagcactgcagcattgaccaggttgatggcaactacagacaccatgagggatctgggagatcagaatttcgactttttattccaagcaacgttgctctatgctcaaattaccaccactgttgcaagagacggatggatcaccagttgtacagatcattatcatattgcctgtaagtcctgtttgagacccatagaagagatcaccctggactcaagtatggactacacgcccccagatgtatcccatgtgctgaagacatggaggaatggggaaggttcgtggggacaagagataaaacagatctatcctttagaagggaattggaagaatttagcacctgctgagcaatcctatcaagtcggcagatgtataggttttctatatggagacttggcgtatagaaaatctactcatgccgaggacagttctctatttcctctatctatacaaggtcgtattagaggtcgaggtttcttaaaagggttgctagacggattaatgagagcaagttgctgccaagtaatacaccggagaagtctggctcatttgaagaggccggccaacgcagtgtacggaggtttgatttacttgattgataaattgagtgtatcacctccattcctttctcttactagatcaggacctattagagacgaattagaaacgattccccacaagatcccaacctcctatccgacaagcaaccgtgatatgggggtgattgtcagaaattacttcaaataccaatgccgtctaattgaaaagggaaaatacagatcacattattcacaattatggttattctcagatgtcttatccatagacttcattggaccattctctatttccaccaccctcttgcaaatcctatacaagccatttttatctgggaaagataagaatgagttgagagagctggcaaatctttcttcattgctaagatcaggagaggggtgggaagacatacatgtgaaattcttcaccaaggacatattattgtgtccagaggaaatcagacatgcttgcaagttcgggattgctaaggataataataaagacatgagctatcccccttggggaagggaatccagagggacaattacaacaatccctgtttattatacgaccaccccttacccaaagatgctagagatgcctccaagaatccaaaatcccctgctgtccggaatcaggttgggccaattaccaactggcgctcattataaaattcggagtatattacatggaatgggaatccattacagggacttcttgagttgtggagacggctccggagggatgactgctgcattactacgagaaaatgtgcatagcagaggaatattcaatagtctgttagaattatcagggtcagtcatgcgaggcgcctctcctgagccccccagtgccctagaaactttaggaggagataaatcgagatgtgtaaatggtgaaacatgttgggaatatccatctgacttatgtgacccaaggacttgggactatttcctccgactcaaagcaggcttggggcttcaaattgatttaattgtaatggatatggaagttcgggattcttctactagcctgaaaattgagacgaatgttagaaattatgtgcaccggattttggatgagcaaggagttttaatctacaagacttatggaacatatatttgtgagagcgaaaagaatgcagtaacaatccttggtcccatgttcaagacggtcgacttagttcaaacagaatttagtagttctcaaacgtctgaagtatatatggtatgtaaaggtttgaagaaattaatcgatgaacccaatcccgattggtcttccatcaatgaatcctggaaaaacctgtacgcattccagtcatcagaacaggaatttgccagagcaaagaaggttagtacatactttaccttgacaggtattccctcccaattcattcctgatccttttgtaaacattgagactatgctacaaatattcggagtacccacgggtgtgtctcatgcggctgccttaaaatcatctgatagacctgcagatttattgaccattagccttttttatatggcgattatatcgtattataacatcaatcatatcagagtaggaccgatacctccgaaccccccatcagatggaattgcacaaaatgtggggatcgctataactggtataagcttttggctgagtttgatggagaaagacattccactatatcaacagtgtttagcagttatccagcaatcattcccgattaggtgggaggctgtttcagtaaaaggaggatacaagcagaagtggagtactagaggtgatgggctcccaaaagatacccgaatttcagactccttggccccaatcgggaactggatcagatctctggaattggtccgaaaccaagttcgtctaaatccattcaatgagatcttgttcaatcagctatgtcgtacagtggataatcatttgaaatggtcaaatttgcgaagaaacacaggaatgattgaatggatcaatagacgaatttcaaaagaagaccggtctatactgatgttgaagagtgacctacacgaggaaaactcttggagagattaaaaaatcatgaggagactccaaactttaagtatgaaaaaaactttgatccttaagaccctcttgtggtttttattttttatctggttttgtggtcttcgtgggtcggcatggcatctccacctcctcgcggtccgacctgggcatccgaaggaggacgtcgtccactcggatggctaagggaggggcccccgcggggctgctaacaaagcccgaaaggaagctgagttggctgctgccaccgctgagcaataactagcataaccccttggggcctctaaacgggtcttgaggggttttttgctgaaaggaggaactatatccggatcgagacctcgatactagtgcggtggagctccagcttttgttccctttagtgagggttaattgcgcgcttggcgtaatcatggtcatagctgtttcctgtgtgaaattgttatccgctcacaattccacacaacatacgagccggaagcataaagtgtaaagcctggggtgcctaatgagtgagctaactcacattaattgcgttgcgctcactgcccgctttccagtcgggaaacctgtcgtgccagctgcattaatgaatcggccaacgcgcggggagaggcggtttgcgtattgggcgctcttccgcttcctcgctcactgactcgctgcgctcggtcgttcggctgcggcgagcggtatcagctcactcaaaggcggtaatacggttatccacagaatcaggggataacgcaggaaagaacatgtgagcaaaaggccagcaaaaggccaggaaccgtaaaaaggccgcgttgctggcgtttttccataggctccgcccccctgacgagcatcacaaaaatcgacgctcaagtcagaggtggcgaaacccgacaggactataaagataccaggcgtttccccctggaagctccctcgtgcgctctcctgttccgaccctgccgcttaccggatacctgtccgcctttctcccttcgggaagcgtggcgctttctcatagctcacgctgtaggtatctcagttcggtgtaggtcgttcgctccaagctgggctgtgtgcacgaaccccccgttcagcccgaccgctgcgccttatccggtaactatcgtcttgagtccaacccggtaagacacgacttatcgccactggcagcagccactggtaacaggattagcagagcgaggtatgtaggcggtgctacagagttcttgaagtggtggcctaactacggctacactagaaggacagtatttggtatctgcgctctgctgaagccagttaccttcggaaaaagagttggtagctcttgatccggcaaacaaaccaccgctggtagcggtggtttttttgtttgcaagcagcagattacgcgcagaaaaaaaggatctcaagaagatcctttgatcttttctacggggtctgacgctcagtggaacgaaaactcacgttaagggattttggtcatgagattatcaaaaaggatcttcacctagatccttttaaattaaaaatgaagttttaaatcaatctaaagtatatatgagtaaacttggtctgacagttaccaatgcttaatcagtgaggcacctatctcagcgatctgtctatttcgttcatccatagttgcctgactccccgtcgtgtagataactacgatacgggagggcttaccatctggccccagtgctgcaatgataccgcgagacccacgctcaccggctccagatttatcagcaataaaccagccagccggaagggccgagcgcagaagtggtcctgcaactttatccgcctccatccagtctattaattgttgccgggaagctagagtaagtagttcgccagttaatagtttgcgcaacgttgttgccattgctacaggcatcgtggtgtcacgctcgtcgtttggtatggcttcattcagctccggttcccaacgatcaaggcgagttacatgatcccccatgttgtgcaaaaaagcggttagctccttcggtcctccgatcgttgtcagaagtaagttggccgcagtgttatcactcatggttatggcagcactgcataattctcttactgtcatgccatccgtaagatgcttttctgtgactggtgagtactcaaccaagtcattctgagaatagtgtatgcggcgaccgagttgctcttgcccggcgtcaatacgggataataccgcgccacatagcagaactttaaaagtgctcatcattggaaaacgttcttcggggcgaaaactctcaaggatcttaccgctgttgagatccagttcgatgtaacccactcgtgcacccaactgatcttcagcatcttttactttcaccagcgtttctgggtgagcaaaaacaggaaggcaaaatgccgcaaaaaagggaataagggcgacacggaaatgttgaatactcatactcttcctttttcaatattattgaagcatttatcagggttattgtctcatgagcggatacatatttgaatgtatttagaaaaataaacaaataggggttccgcgcacatttccccgaaaagtgccac

SEQ ID NO: 16 - protein, 1536 aa, Vesicular stomatitis virus
ATGAAGTGCCTTTTGTACTTAGCCTTTTTATTCATTGGGGTGAATTGCAAGTTCACCATAGTTTTTCCACACAACCAAAAAGGAAACTGGAAAAATGTTCCTTCTAATTACCATTATTGCCCGTCAAGCTCAGATTTAAATTGGCATAATGACTTAATAGGCACAGCCTTACAAGTCAAAATGCCCAAGAGTCACAAGGCTATTCAAGCAGACGGTTGGATGTGTCATGCTTCCAAATGGGTCACTACTTGTGATTTCCGCTGGTATGGACCGAAGTATATAACACATTCCATCCGATCCTTCACTCCATCTGTAGAACAATGCAAGGAAAGCATTGAACAAACGAAACAAGGAACTTGGCTGAATCCAGGCTTCCCTCCTCAAAGTTGTGGATATGCAACTGTGACGGATGCCGAAGCAGTGATTGTCCAGGTGACTCCTCACCATGTGCTGGTTGATGAATACACAGGAGAATGGGTTGATTCACAGTTCATCAACGGAAAATGCAGCAATTACATATGCCCCACTGTCCATAACTCTACAACCTGGCATTCTGACTATAAGGTCAAAGGGCTATGTGATTCTAACCTCATTTCCATGGACATCACCTTCTTCTCAGAGGACGGAGAGCTATCATCCCTGGGAAAGGAGGGCACAGGGTTCAGAAGTAACTACTTTGCTTATGAAACTGGAGGCAAGGCCTGCAAAATGCAATACTGCAAGCATTGGGGAGTCAGACTCCCATCAGGTGTCTGGTTCGAGATGGCTGATAAGGATCTCTTTGCTGCAGCCAGATTCCCTGAATGCCCAGAAGGGTCAAGTATCTCTGCTCCATCTCAGACCTCAGTGGATGTAAGTCTAATTCAGGACGTTGAGAGGATCTTGGATTATTCCCTCTGCCAAGAAACCTGGAGCAAAATCAGAGCGGGTCTTCCAATCTCTCCAGTGGATCTCAGCTATCTTGCTCCTAAAAACCCAGGAACCGGTCCTGCTTTCACCATAATCAATGGTACCCTAAAATACTTTGAGACCAGATACATCAGAGTCGATATTGCTGCTCCAATCCTCTCAAGAATGGTCGGAATGATCAGTGGAACTACCACAGAAAGGGAACTGTGGGATGACTGGGCACCATATGAAGACGTGGAAATTGGACCCAATGGAGTTCTGAGGACCAGTTCAGGATATAAGTTTCCTTTATACATGATTGGACATGGTATGTTGGACTCCGATCTTCATCTTAGCTCAAAGGCTCAGGTGTTCGAACATCCTCACATTCAAGACGCTGCTTCGCAACTTCCTGATGATGAGAGTTTATTTTTTGGTGATACTGGGCTATCCAAAAATCCAATCGAGCTTGTAGAAGGTTGGTTCAGTAGTTGGAAAAGCTCTATTGCCTCTTTTTTCTTTATCATAGGGTTAATCATTGGACTATTCTTGGTTCTCCGAGTTGGTATCCATCTTTGCATTAAATTAAAGCACACCAAGAAAAGACAGATTTATACAGACATAGAGATGAACCGACTTGGAAAGTAA